European Patent Specification EP 3 481 855 B1, published September 6, 2023. Title: LONG-ACTING COAGULATION FACTORS AND METHODS OF PRODUCING SAME. Applicant: OPKO BIOLOGICS LTD. HERSHKOVITZ, Oren MOSCHCOVICH, Laura. The sequence listing filed with the application follows.

SEQUENCE LISTING (15 sequences)

SEQ ID NO: 1 - DNA, 1356 bp, Homo sapiens
ctcgaggacatggtctcccaggccctcaggctcctctgccttctgcttgggcttcagggctgcctggctgcagtcttcgtaacccaggaggaagcccacggcgtcctgcaccggcgccggcgcgccaacgcgttcctggaggagctgcggccgggctccctggagagggagtgcaaggaggagcagtgctccttcgaggaggcccgggagatcttcaaggacgcggagaggacgaagctgttctggatttcttacagtgatggggaccagtgtgcctcaagtccatgccagaatgggggctcctgcaaggaccagctccagtcctatatctgcttctgcctccctgccttcgagggccggaactgtgagacgcacaaggatgaccagctgatctgtgtgaacgagaacggcggctgtgagcagtactgcagtgaccacacgggcaccaagcgctcctgtcggtgccacgaggggtactctctgctggcagacggggtgtcctgcacacccacagttgaatatccatgtggaaaaatacctattctagaaaaaagaaatgccagcaaaccccaaggccgaattgtggggggcaaggtgtgccccaaaggggagtgtccatggcaggtcctgttgttggtgaatggagctcagttgtgtggggggaccctgatcaacaccatctgggtggtctccgcggcccactgtttcgacaaaatcaagaactggaggaacctgatcgcggtgctgggcgagcacgacctcagcgagcacgacggggatgagcagagccggcgggtggcgcaggtcatcatccccagcacgtacgtcccgggcaccaccaaccacgacatcgcgctgctccgcctgcaccagcccgtggtcctcactgaccatgtggtgcccctctgcctgcccgaacggacgttctctgagaggacgctggccttcgtgcgcttctcattggtcagcggctggggccagctgctggaccgtggcgccacggccctggagctcatggtcctcaacgtgccccggctgatgacccaggactgcctgcagcagtcacggaaggtgggagactccccaaatatcacggagtacatgttctgtgccggctactcggatggcagcaaggactcctgcaagggggacagtggaggcccacatgccacccactaccggggcacgtggtacctgacgggcatcgtcagctggggccagggctgcgcaaccgtgggccactttggggtgtacaccagggtctcccagtacatcgagtggctgcaaaagctcatgcgctcagagccacgcccaggagtcctcctgcgagccccatttccctgaggatgcggccgc

SEQ ID NO: 2 - protein, 444 aa, Homo sapiens
MVSQALRLLCLLLGLQGCLAAVFVTQEEAHGVLHRRRRANAFLEELRPGSLERECKEEQCSFEEAREIFKDAERTKLFWISYSDGDQCASSPCQNGGSCKDQLQSYICFCLPAFEGRNCETHKDDQLICVNENGGCEQYCSDHTGTKRSCRCHEGYSLLADGVSCTPTVEYPCGKIPILEKRNASKPQGRIVGGKVCPKGECPWQVLLLVNGAQLCGGTLINTIWVVSAAHCFDKIKNWRNLIAVLGEHDLSEHDGDEQSRRVAQVIIPSTYVPGTTNHDIALLRLHQPVVLTDHVVPLCLPERTFSERTLAFVRFSLVSGWGQLLDRGATALELMVLNVPRLMTQDCLQQSRKVGDSPNITEYMFCAGYSDGSKDSCKGDSGGPHATHYRGTWYLTGIVSWGQGCATVGHFGVYTRVSQYIEWLQKLMRSEPRPGVLLRAPFP

SEQ ID NO: 3 - protein, 448 aa, Homo sapiens
MVSQALRLLCLLLGLQGCLAAVFVTQEEAHGVLHRRRRANAFLEELRPGSLERECKEEQCSFEEAREIFKDAERTKLFWISYSDGDQCASSPCQNGGSCKDQLQSYICFCLPAFEGRNCETHKDDQLICVNENGGCEQYCSDHTGTKRSCRCHEGYSLLADGVSCTPTVEYPCGKIPILEKRNASKPQGRIVGGKVCPKGECPWQVLLLVNGAQLCGGTLINTIWVVSAAHCFDKIKNWRNLIAVLGEHDLSEHDGDEQSRRVAQVIIPSTYVPGTTNHDIALLRLHQPVVLTDHVVPLCLPERTFSERTLAFVRFSLVSGWGQLLDRGATALELMVLNVPRLMTQDCLQQSRKVGDSPNITEYMFCAGYSDGSKDSCKGDSGGPHATHYRGTWYLTGIVSWGQGCATVGHFGVYTRVSQYIEWLQKLMRSEPRPGVLLRAPFPGCGR

SEQ ID NO: 4 - DNA, 1621 bp, Artificial Sequence
  CTP-Modified Factor VII
ctcgaggacatggtctcccaggccctcaggctcctctgccttctgcttgggcttcagggctgcctggctgcagtcttcgtaacccaggaggaagcccacggcgtcctgcaccggcgccggcgcgccaacgcgttcctggaggagctgcggccgggctccctggagagggagtgcaaggaggagcagtgctccttcgaggaggcccgggagatcttcaaggacgcggagaggacgaagctgttctggatttcttacagtgatggggaccagtgtgcctcaagtccatgccagaatgggggctcctgcaaggaccagctccagtcctatatctgcttctgcctccctgccttcgagggccggaactgtgagacgcacaaggatgaccagctgatctgtgtgaacgagaacggcggctgtgagcagtactgcagtgaccacacgggcaccaagcgctcctgtcggtgccacgaggggtactctctgctggcagacggggtgtcctgcacacccacagttgaatatccatgtggaaaaatacctattctagaaaaaagaaatgccagcaaaccccaaggccgaattgtggggggcaaggtgtgccccaaaggggagtgtccatggcaggtcctgttgttggtgaatggagctcagttgtgtggggggaccctgatcaacaccatctgggtggtctccgcggcccactgtttcgacaaaatcaagaactggaggaacctgatcgcggtgctgggcgagcacgacctcagcgagcacgacggggatgagcagagccggcgggtggcgcaggtcatcatccccagcacgtacgtcccgggcaccaccaaccacgacatcgcgctgctccgcctgcaccagcccgtggtcctcactgaccatgtggtgcccctctgcctgcccgaacggacgttctctgagaggacgctggccttcgtgcgcttctcattggtcagcggctggggccagctgctggaccgtggcgccacggccctggagctcatggtcctcaacgtgccccggctgatgacccaggactgcctgcagcagtcacggaaggtgggagactccccaaatatcacggagtacatgttctgtgccggctactcggatggcagcaaggactcctgcaagggggacagtggaggcccacatgccacccactaccggggcacgtggtacctgaccggcatcgtgagctggggccagggctgcgccaccgtgggccacttcggcgtgtacaccagggtgtcccagtacatcgagtggctgcagaaactgatgagaagcgagcccagacccggcgtgctgctgagagcccccttccccagcagcagctccaaggcccctccccctagcctgcccagccctagcagactgcctgggcccagtgacacccctatcctgcctcagtccagctccagcaaggccccaccccctagcctgccttctccttctcggctgcctggccccagcgatactccaattctgccccagtcctccagcagtaaggctccccctccatctctgccatcccccagcagactgccaggcccttctgatacacccatcctcccacagtgatgaggatccgcggccgcttaattaa

SEQ ID NO: 5 - protein, 528 aa, Artificial Sequence
  CTP-Modified Factor VII
MVSQALRLLCLLLGLQGCLAAVFVTQEEAHGVLHRRRRANAFLEELRPGSLERECKEEQCSFEEAREIFKDAERTKLFWISYSDGDQCASSPCQNGGSCKDQLQSYICFCLPAFEGRNCETHKDDQLICVNENGGCEQYCSDHTGTKRSCRCHEGYSLLADGVSCTPTVEYPCGKIPILEKRNASKPQGRIVGGKVCPKGECPWQVLLLVNGAQLCGGTLINTIWVVSAAHCFDKIKNWRNLIAVLGEHDLSEHDGDEQSRRVAQVIIPSTYVPGTTNHDIALLRLHQPVVLTDHVVPLCLPERTFSERTLAFVRFSLVSGWGQLLDRGATALELMVLNVPRLMTQDCLQQSRKVGDSPNITEYMFCAGYSDGSKDSCKGDSGGPHATHYRGTWYLTGIVSWGQGCATVGHFGVYTRVSQYIEWLQKLMRSEPRPGVLLRAPFPSSSSKAPPPSLPSPSRLPGPSDTPILPQSSSSKAPPPSLPSPSRLPGPSDTPILPQSSSSKAPPPSLPSPSRLPGPSDTPILPQ

SEQ ID NO: 6 - protein, 38 aa, Artificial Sequence
  Signal Sequence
MVSQALRLLCLLLGLQGCLAAVFVTQEEAHGVLHRRRR

SEQ ID NO: 7 - protein, 490 aa, Artificial Sequence
  CTP- Modified Factor VII
ANAFLEELRPGSLERECKEEQCSFEEAREIFKDAERTKLFWISYSDGDQCASSPCQNGGSCKDQLQSYICFCLPAFEGRNCETHKDDQLICVNENGGCEQYCSDHTGTKRSCRCHEGYSLLADGVSCTPTVEYPCGKIPILEKRNASKPQGRIVGGKVCPKGECPWQVLLLVNGAQLCGGTLINTIWVVSAAHCFDKIKNWRNLIAVLGEHDLSEHDGDEQSRRVAQVIIPSTYVPGTTNHDIALLRLHQPVVLTDHVVPLCLPERTFSERTLAFVRFSLVSGWGQLLDRGATALELMVLNVPRLMTQDCLQQSRKVGDSPNITEYMFCAGYSDGSKDSCKGDSGGPHATHYRGTWYLTGIVSWGQGCATVGHFGVYTRVSQYIEWLQKLMRSEPRPGVLLRAPFPSSSSKAPPPSLPSPSRLPGPSDTPILPQSSSSKAPPPSLPSPSRLPGPSDTPILPQSSSSKAPPPSLPSPSRLPGPSDTPILPQ

SEQ ID NO: 8 - protein, 152 aa, Artificial Sequence [sequence omitted]

SEQ ID NO: 9 - protein, 338 aa, Artificial Sequence
  CTP-Modified Factor VII - Heavy Chain
IVGGKVCPKGECPWQVLLLVNGAQLCGGTLINTIWVVSAAHCFDKIKNWRNLIAVLGEHDLSEHDGDEQSRRVAQVIIPSTYVPGTTNHDIALLRLHQPVVLTDHVVPLCLPERTFSERTLAFVRFSLVSGWGQLLDRGATALELMVLNVPRLMTQDCLQQSRKVGDSPNITEYMFCAGYSDGSKDSCKGDSGGPHATHYRGTWYLTGIVSWGQGCATVGHFGVYTRVSQYIEWLQKLMRSEPRPGVLLRAPFPSSSSKAPPPSLPSPSRLPGPSDTPILPQSSSSKAPPPSLPSPSRLPGPSDTPILPQSSSSKAPPPSLPSPSRLPGPSDTPILPQ

SEQ ID NO: 10 - DNA, 2413 bp, Homo sapiens
tctagagtcgaccccgccatggagctgaggccctggttgctatgggtggtagcagcaacaggaaccttggtcctgctagcagctgatgctcagggccagaaggtcttcaccaacacgtgggctgtgcgcatccctggaggcccagcggtggccaacagtgtggcacggaagcatgggttcctcaacctgggccagatcttcggggactattaccacttctggcatcgaggagtgacgaagcggtccctgtcgcctcaccgcccgcggcacagccggctgcagagggagcctcaagtacagtggctggaacagcaggtggcaaagcgacggactaaacgggacgtgtaccaggagcccacagaccccaagtttcctcagcagtggtacctgtctggtgtcactcagcgggacctgaatgtgaaggcggcctgggcgcagggctacacagggcacggcattgtggtctccattctggacgatggcatcgagaagaaccacccggacttggcaggcaattatgatcctggggccagttttgatgtcaatgaccaggaccctgacccccagcctcggtacacacagatgaatgacaacaggcacggcacacggtgtgcgggggaagtggctgcggtggccaacaacggtgtctgtggtgtaggtgtggcctacaacgcccgcattggaggggtgcgcatgctggatggcgaggtgacagatgcagtggaggcacgctcgctgggcctgaaccccaaccacatccacatctacagtgccagctggggccccgaggatgacggcaagacagtggatgggccagcccgcctcgccgaggaggccttcttccgtggggttagccagggccgaggggggctgggctccatctttgtctgggcctcggggaacgggggccgggaacatgacagctgcaactgcgacggctacaccaacagtatctacacgctgtccatcagcagcgccacgcagtttggcaacgtgccgtggtacagcgaggcctgctcgtccacactggccacgacctacagcagtggcaaccagaatgagaagcagatcgtgacgactgacttgcggcagaagtgcacggagtctcacacgggcacctcagcctctgcccccttagcagccggcatcattgctctcaccctggaggccaataagaacctcacatggcgggacatgcaacacctggtggtacagacctcgaagccagcccacctcaatgccaacgactgggccaccaatggtgtgggccggaaagtgagccactcatatggctacgggcttttggacgcaggcgccatggtggccctggcccagaattggaccacagtggccccccagcggaagtgcatcatcgacatcctcaccgagcccaaagacatcgggaaacggctcgaggtgcggaagaccgtgaccgcgtgcctgggcgagcccaaccacatcactcggctggagcacgctcaggcgcggctcaccctgtcctataatcgccgtggcgacctggccatccacctggtcagccccatgggcacccgctccaccctgctggcagccaggccacatgactactccgcagatgggtttaatgactgggccttcatgacaactcattcctgggatgaggatccctctggcgagtgggtcctagagattgaaaacaccagcgaagccaacaactatgggacgctgaccaagttcaccctcgtactctatggcaccgcccctgaggggctgcccgtacctccagaaagcagtggctgcaagaccctcacgtccagtcaggcctgtgtggtgtgcgaggaaggcttctccctgcaccagaagagctgtgtccagcactgccctccaggcttcgccccccaagtcctcgatacgcactatagcaccgagaatgacgtggagaccatccgggccagcgtctgcgccccctgccacgcctcatgtgccacatgccaggggccggccctgacagactgcctcagctgccccagccacgcctccttggaccctgtggagcagacttgctcccggcaaagccagagcagccgagagtccccgccacagcagcagccacctcggctgcccccggaggtggaggcggggcaacggctgcgggcagggctgctgccctcacacctgcctgaggtggtggccggcctcagctgcgccttcatcgtgctggtcttcgtcactgtcttcctggtcctgcagctgcgctctggctttagttttcggggggtgaaggtgtacaccatggaccgtggcctcatctcctacaaggggctgccccctgaagcctggcaggaggagtgcccgtctgactcagaagaggacgagggccggggcgagaggaccgcctttatcaaagaccagagcgccctctgaacgcggccgc

SEQ ID NO: 11 - protein, 793 aa, Homo sapiens
MELRPWLLWVVAATGTLVLLAADAQGQKVFTNTWAVRIPGGPAVANSVARKHGFLNLGQIFGDYYHFWHRGVTKRSLSPHRPRHSRLQREPQVQWLEQQVAKRRTKRDVYQEPTDPKFPQQWYLSGVTQRDLNVKAAWAQGYTGHGIVVSILDDGIEKNHPDLAGNYDPGASFDVNDQDPDPQPRYTQMNDNRHGTRCAGEVAAVANNGVCGVGVAYNARIGGVRMLDGEVTDAVEARSLGLNPNHIHIYSASWGPEDDGKTVDGPARLAEEAFFRGVSQGRGGLGSIFVWASGNGGREHDSCNCDGYTNSIYTLSISSATQFGNVPWYSEACSSTLATTYSSGNQNEKQIVTTDLRQKCTESHTGTSASAPLAAGIIALTLEANKNLTWRDMQHLVVQTSKPAHLNANDWATNGVGRKVSHSYGYGLLDAGAMVALAQNWTTVAPQRKCIIDILTEPKDIGKRLEVRKTVTACLGEPNHITRLEHAQARLTLSYNRRGDLAIHLVSPMGTRSTLLAARPHDYSADGFNDWAFMTTHSWDEDPSGEWVLEIENTSEANNYGTLTKFTLVLYGTAPEGLPVPPESSGCKTLTSSQACVVCEEGFSLHQKSCVQHCPPGFAPQVLDTHYSTENDVETIRASVCAPCHASCATCQGPALTDCLSCPSHASLDPVEQTCSRQSQSSRESPPQQQPPRLPPEVEAGQRLRAGLLPSHLPEVVAGLSCAFIVLVFVTVFLVLQLRSGFSFRGVKVYTMDRGLISYKGLPPEAWQEECPSDSEEDEGRGERTAFIKDQSA

SEQ ID NO: 12 - protein, 32 aa, Homo sapiens
DPRFQDSSSSKAPPPSLPSPSRLPGPSDTPIL

SEQ ID NO: 13 - protein, 28 aa, Homo sapiens
SSSSKAPPPSLPSPSRLPGPSDTPILPQ

SEQ ID NO: 14 - protein, 12 aa, Homo sapiens
SSSSKAPPPSLP

SEQ ID NO: 15 - protein, 10 aa, Homo sapiens
SSSSKAPPPS